European Patent Specification EP 3 727 470 B1, published November 20, 2024. Title: PEPTIDE NUCLEIC ACID CONJUGATES. Applicant: VENTANA MEDICAL SYSTEMS, INC. The sequence listing filed with the application follows.

SEQUENCE LISTING (21 sequences)

SEQ ID NO: 1 - DNA, 15 bp, Artificial Sequence
  Synthetic: Synthetic PNA sequence
gtcaaccatcttcag

SEQ ID NO: 2 - DNA, 15 bp, Artificial Sequence
  Synthetic: Synthetic PNA sequence
ttagtccaactggca

SEQ ID NO: 3 - DNA, 15 bp, Artificial Sequence
  Synthetic: Synthetic PNA sequence
cattcaaatccccga

SEQ ID NO: 4 - DNA, 10 bp, Artificial Sequence
  Synthetic: Synthetic PNA sequence
ccatcttcag

SEQ ID NO: 5 - DNA, 10 bp, Artificial Sequence
  Synthetic: Synthetic PNA sequence
ttagtccaac

SEQ ID NO: 6 - DNA, 10 bp, Artificial Sequence
  Synthetic: Synthetic PNA sequence
cattcaaatc

SEQ ID NO: 7 - DNA, 10 bp, Artificial Sequence
  Synthetic: Synthetic PNA sequence
catcctgccg

SEQ ID NO: 8 - DNA, 15 bp, Artificial Sequence
  Synthetic: Synthetic PNA conjugate
  modified_base (1)..(1): Biotin-O on 5' end
  modified_base (15)..(15): Lys(C6SH) on 3' end
gtcaaccatcttcag

SEQ ID NO: 9 - DNA, 15 bp, Artificial Sequence
  Synthetic: Synthetic PNA conjugate
  modified_base (1)..(1): Biotin-O on 5' end
  modified_base (15)..(15): Lys(C6SH) on 3' end
ttagtccaactggca

SEQ ID NO: 10 - DNA, 15 bp, Artificial Sequence
  Synthetic: Synthetic PNA conjugate
  modified_base (1)..(1): Biotin-O on 5' end
  modified_base (15)..(15): PL-Lys(C6SH), PL: Photocleavable Linker on 3' end
cattcaaatccccga

SEQ ID NO: 11 - DNA, 15 bp, Artificial Sequence
  Synthetic: Synthetic PNA conjugate
  modified_base (1)..(1): Biotin-O on 5' end
  modified_base (15)..(15): Lys(C6SH) on 3' end
ctgaagatggtttac

SEQ ID NO: 12 - DNA, 15 bp, Artificial Sequence
  Synthetic: Synthetic PNA conjugate
  modified_base (1)..(1): Alexa488-O on 5' end
  modified_base (15)..(15): Lys(C6SH) on 3' end
catcctgccgctatg

SEQ ID NO: 13 - DNA, 15 bp, Artificial Sequence
  Synthetic: Synthetic PNA conjugate
  modified_base (1)..(1): Biotin-O on 5' end
  modified_base (15)..(15): Arg-O-Cys on 3' end
gtcaaccatcttcag

SEQ ID NO: 14 - DNA, 15 bp, Artificial Sequence
  Synthetic: Synthetic PNA conjugate
  modified_base (1)..(1): Biotin-O on 5' end
  modified_base (15)..(15): Lys(eg3-N3) on 3' end
gtcaaccatcttcag

SEQ ID NO: 15 - DNA, 15 bp, Artificial Sequence
  Synthetic: Synthetic PNA conjugate
  modified_base (1)..(1): Biotin-O on 5' end
  modified_base (15)..(15): Lys(SMCC), SMCC: maleimide moeity on 3' end
gtcaaccatcttcag

SEQ ID NO: 16 - DNA, 15 bp, Artificial Sequence
  Synthetic: Synthetic DNA conjugate
  modified_base (15)..(15): Rhodamine on 3' end
ctgaagatggttgac

SEQ ID NO: 17 - DNA, 15 bp, Artificial Sequence
  Synthetic: Synthetic DNA conjugate
  modified_base (1)..(1): FAM on 5' end
ctgaagatggttgac

SEQ ID NO: 18 - DNA, 15 bp, Artificial Sequence
  Synthetic: Synthetic DNA conjugate
  modified_base (15)..(15): DIG on 3' end
ctgaagatggttgac

SEQ ID NO: 19 - DNA, 10 bp, Artificial Sequence
  Synthetic: Synthetic PNA conjugate
  modified_base (1)..(1): Biotin-O on 5' end
  modified_base (10)..(10): Lys(SMCC) on 3' end, SMCC: maleimide moiety
ccatcttcag

SEQ ID NO: 20 - DNA, 10 bp, Artificial Sequence
  Synthetic: Synthetic PNA conjugate
  modified_base (1)..(1): Biotin-O on 5' end
  modified_base (10)..(10): Lys(SMCC) on 3' end, SMCC: maleimide moity
ttagtccaac

SEQ ID NO: 21 - DNA, 10 bp, Artificial Sequence
  Synthetic: Synthetic PNA conjugate
  modified_base (1)..(1): Biotin-O on 5' end
  modified_base (10)..(10): Lys(C6SH) on 3' end
ccatcttcag